European Patent Application EP 4 755 909 A1, published June 10, 2026. Title: A CONJUGATE OF MODIFIED FUSION PROTEIN AND A SCFV, AND THE USE THEREOF. Applicant: 주식회사 파노로스바이오사이언스. Application KR. The sequence listing filed with the application follows.

SEQUENCE LISTING (79 sequences)

SEQ ID NO: 1 - protein, 692 aa, synthetic construct
QVQLQESGPGLVKPSETLSITCTVSGFSLSNYDISWIRQPPGKGLEWLGVIWTGGATNYNPALKSRLTISRDNSKNQVSLKMSSVTAADTAVYYCVRDSNYRYDEPFTYWGQGTLVTVSSGGGGSGGGGSGGGGSGGGGSGGGGSEIVLTQSPDTLSVTPKEKVTLTCRASQSIGTNIHWFQQKPGQSPKLLIKYASESISGVPSRFSGSGSGTDFTLTINSVEAEDAATYYCQQSNSWPYTFGQGTKLEIKRTVGGGGSEFGRPFVEMYSEIPEIIHMTEGRELVIPCRVTSPNITVTLKKFPLDTLIPDGKRIIWDSRKGFIISNATYKEIGLLTCEATVNGHLYKTNYLTHRQTNTIIDVQISTPSPVTLLRGHTLVLNCTATTPLNTRVQMTWSYPDEKNKNASVRRRIDQSNSHANIFYSVLTIDKMQNKDKGLYTCRVRSGPSFKSVNTSVHIYDKALEDKTHTCPPCPAPELLGGPSVFLFPPKPKDTLMISRTPEVTCVVVDVSHEDPEVKFNWYVDGVEVHNAKTKPREEQYNSTYRVVSVLTVLHQDWLNGKEYKCKVSNKALPAPIEKTISKAKGQPREPQVYTLPPSREEMTKNQVSLTCLVKGFYPSDIAVEWESNGQPENNYKTTPPVLDSDGSFFLYSKLTVDKSRWQQGNVFSCSVMHEALHNHYTQKSLSLSPGK

SEQ ID NO: 2 - protein, 692 aa, synthetic construct
EIVLTQSPDTLSVTPKEKVTLTCRASQSIGTNIHWFQQKPGQSPKLLIKYASESISGVPSRFSGSGSGTDFTLTINSVEAEDAATYYCQQSNSWPYTFGQGTKLEIKRTVGGGGSGGGGSGGGGSGGGGSGGGGSQVQLQESGPGLVKPSETLSITCTVSGFSLSNYDISWIRQPPGKGLEWLGVIWTGGATNYNPALKSRLTISRDNSKNQVSLKMSSVTAADTAVYYCVRDSNYRYDEPFTYWGQGTLVTVSSGGGGSEFGRPFVEMYSEIPEIIHMTEGRELVIPCRVTSPNITVTLKKFPLDTLIPDGKRIIWDSRKGFIISNATYKEIGLLTCEATVNGHLYKTNYLTHRQTNTIIDVQISTPSPVTLLRGHTLVLNCTATTPLNTRVQMTWSYPDEKNKNASVRRRIDQSNSHANIFYSVLTIDKMQNKDKGLYTCRVRSGPSFKSVNTSVHIYDKALEDKTHTCPPCPAPELLGGPSVFLFPPKPKDTLMISRTPEVTCVVVDVSHEDPEVKFNWYVDGVEVHNAKTKPREEQYNSTYRVVSVLTVLHQDWLNGKEYKCKVSNKALPAPIEKTISKAKGQPREPQVYTLPPSREEMTKNQVSLTCLVKGFYPSDIAVEWESNGQPENNYKTTPPVLDSDGSFFLYSKLTVDKSRWQQGNVFSCSVMHEALHNHYTQKSLSLSPGK

SEQ ID NO: 3 - protein, 497 aa, synthetic construct
QVQLQESGPGLVKPSETLSITCTVSGFSLSNYDISWIRQPPGKGLEWLGVIWTGGATNYNPALKSRLTISRDNSKNQVSLKMSSVTAADTAVYYCVRDSNYRYDEPFTYWGQGTLVTVSSGGGGSGGGGSGGGGSGGGGSGGGGSEIVLTQSPDTLSVTPKEKVTLTCRASQSIGTNIHWFQQKPGQSPKLLIKYASESISGVPSRFSGSGSGTDFTLTINSVEAEDAATYYCQQSNSWPYTFGQGTKLEIKRTVGGGGSGGGGSGGGGSDKTHTCPPCPAPELLGGPSVFLFPPKPKDTLMISRTPEVTCVVVDVSHEDPEVKFNWYVDGVEVHNAKTKPREEQYNSTYRVVSVLTVLHQDWLNGKEYKCKVSNKALPAPIEKTISKAKGQPREPQVYTLPPSREEMTKNQVSLTCLVKGFYPSDIAVEWESNGQPENNYKTTPPVLDSDGSFFLYSKLTVDKSRWQQGNVFSCSVMHEALHNHYTQKSLSLSPGK

SEQ ID NO: 4 - protein, 702 aa, synthetic construct
EFGRPFVEMYSEIPEIIHMTEGRELVIPCRVTSPNITVTLKKFPLDTLIPDGKRIIWDSRKGFIISNATYKEIGLLTCEATVNGHLYKTNYLTHRQTNTIIDVQISTPSPVTLLRGHTLVLNCTATTPLNTRVQMTWSYPDEKNKNASVRRRIDQSNSHANIFYSVLTIDKMQNKDKGLYTCRVRSGPSFKSVNTSVHIYDKALEDKTHTCPPCPAPELLGGPSVFLFPPKPKDTLMISRTPEVTCVVVDVSHEDPEVKFNWYVDGVEVHNAKTKPREEQYNSTYRVVSVLTVLHQDWLNGKEYKCKVSNKALPAPIEKTISKAKGQPREPQVYTLPPSREEMTKNQVSLTCLVKGFYPSDIAVEWESNGQPENNYKTTPPVLDSDGSFFLYSKLTVDKSRWQQGNVFSCSVMHEALHNHYTQKSLSLSPGKGGGGSGGGGSGGGGSQVQLQESGPGLVKPSETLSITCTVSGFSLSNYDISWIRQPPGKGLEWLGVIWTGGATNYNPALKSRLTISRDNSKNQVSLKMSSVTAADTAVYYCVRDSNYRYDEPFTYWGQGTLVTVSSGGGGSGGGGSGGGGSGGGGSGGGGSEIVLTQSPDTLSVTPKEKVTLTCRASQSIGTNIHWFQQKPGQSPKLLIKYASESISGVPSRFSGSGSGTDFTLTINSVEAEDAATYYCQQSNSWPYTFGQGTKLEIKRTV

SEQ ID NO: 5 - protein, 708 aa, synthetic construct
QVQLQESGPGLVKPSETLSITCTVSGFSLSNYDISWIRQPPGKGLEWLGVIWTGGATNYNPALKSRLTISRDNSKNQVSLKMSSVTAADTAVYYCVRDSNYRYDEPFTYWGQGTLVTVSSGGGGSGGGGSGGGGSGGGGSEIVLTQSPDTLSVTPKEKVTLTCRASQSIGTNIHWFQQKPGQSPKLLIKYASESISGVPSRFSGSGSGTDFTLTINSVEAEDAATYYCQQSNSWPYTFGQGTKLEIKRGSGGGGSGGGGSGGGGSGGGGSGRPFVEMYSEIPEIIHMTEGRELVIPCRVTSPNITVTLKKFPLDTLIPDGKRIIWDSRKGFIISNATYKEIGLLTCEATVNGHLYKTNYLTHRQTNTIIDVQISTPSPVTLCRGHTLVLNCTATTPANTRVQMTWSYPDEKNKNASVRRRIDQSNSHANIFYSVLTIDGMTNSDQGLYTCRVRSGPSFKSVNTSVHIYDCGSSGGSSGEPKSDATPTCPPCPAPELLGGPSVFLFPPKPKDTLMISRTPEVTCVVVDVSHEDPEVKFNWYVDGVEVHNAKTKPREEQYNSTYRVVSVLTVLHQDWLNGKEYKCKVSNKALPAPIEKTISKAKGQPREPQVYTLPPSRDELTKNQVSLTCLVKGFYPSDIAVEWESNGQPENNYKTTPPVLDSDGSFFLYSKLTVDKSRWQQGNVFSCSVMHEALHNHYTQKSLSLSPG

SEQ ID NO: 6 - protein, 698 aa, synthetic construct
QVQLQESGPGLVKPSETLSITCTVSGFSLSNYDISWIRQPPGKGLEWLGVIWTGGATNYNPALKSRLTISRDNSKNQVSLKMSSVTAADTAVYYCVRDSNYRYDEPFTYWGQGTLVTVSSGGGGSGGGGSGGGGSGGGGSEIVLTQSPDTLSVTPKEKVTLTCRASQSIGTNIHWFQQKPGQSPKLLIKYASESISGVPSRFSGSGSGTDFTLTINSVEAEDAATYYCQQSNSWPYTFGQGTKLEIKRGGGGSGGGGSDTGRPFVEMYSEIPEIIHMTEGRELVIPCRVTSPNITVTLKKFPLDTLIPDGKRIIWDSRKGFIISNATYKEIGLLTCEATVNGHLYKTNYLTHRQTNTIIDVQISTPSPVTLCRGHTLVLNCTATTPANTRVQMTWSYPDEKNKNASVRRRIDQSNSHANIFYSVLTIDGMTNSDQGLYTCRVRSGPSFKSVNTSVHIYDCGSSGGSSGEPKSDATPTCPPCPAPELLGGPSVFLFPPKPKDTLMISRTPEVTCVVVDVSHEDPEVKFNWYVDGVEVHNAKTKPREEQYNSTYRVVSVLTVLHQDWLNGKEYKCKVSNKALPAPIEKTISKAKGQPREPQVYTLPPSRDELTKNQVSLTCLVKGFYPSDIAVEWESNGQPENNYKTTPPVLDSDGSFFLYSKLTVDKSRWQQGNVFSCSVMHEALHNHYTQKSLSLSPG

SEQ ID NO: 7 - protein, 720 aa, synthetic construct
  MUTAGEN 494: note = The residue of Serine was mutated to Cysteine
QVQLQESGPGLVKPSETLSITCTVSGFSLSNYDISWIRQPPGKGLEWLGVIWTGGATNYNPALKSRLTISRDNSKNQVSLKMSSVTAADTAVYYCVRDSNYRYDEPFTYWGQGTLVTVSSGGGGSGGGGSGGGGSGGGGSEIVLTQSPDTLSVTPKEKVTLTCRASQSIGTNIHWFQQKPGQSPKLLIKYASESISGVPSRFSGSGSGTDFTLTINSVEAEDAATYYCQQSNSWPYTFGQGTKLEIKRGSGGGGSGGGGSGGGGSGGGGSGRPFVEMYSEIPEIIHMTEGRELVIPCRVTSPNITVTLKKFPLDTLIPDGKRIIWDSRKGFIISNATYKEIGLLTCEATVNGHLYKTNYLTHRQTNTIIDVQISTPSPVTLCRGHTLVLNCTATTPANTRVQMTWSYPDEKNKNASVRRRIDQSNSHANIFYSVLTIDGMTNSDQGLYTCRVRSGPSFKSVNTSVHIYDCSNTGSGGEEKKKEKEKEEQEERSCDTPPTCPPCPAPELLGGPSVFLFPPKPKDTLMISRTPEVTCVVVDVSHEDPEVKFNWYVDGVEVHNAKTKPREEQYNSTYRVVSVLTVLHQDWLNGKEYKCKVSNKALPAPIEKTISKAKGQPREPQVYTLPPSRDELTKNQVSLTCLVKGFYPSDIAVEWESNGQPENNYKTTPPVLDSDGSFFLYSKLTVDKSRWQQGNVFSCSVMHEALHNHYTQKSLSLSPG

SEQ ID NO: 8 - protein, 715 aa, synthetic construct
QVQLQESGPGLVKPSETLSITCTVSGFSLSNYDISWIRQPPGKGLEWLGVIWTGGATNYNPALKSRLTISRDNSKNQVSLKMSSVTAADTAVYYCVRDSNYRYDEPFTYWGQGTLVTVSSGGGGSGGGGSGGGGSGGGGSEIVLTQSPDTLSVTPKEKVTLTCRASQSIGTNIHWFQQKPGQSPKLLIKYASESISGVPSRFSGSGSGTDFTLTINSVEAEDAATYYCQQSNSWPYTFGQGTKLEIKRGSGGGGSGGGGSGGGGSGGGGSGRPFVEMYSEIPEIIHMTEGRELVIPCRVTSPNITVTLKKFPLDTLIPDGKRIIWDSRKGFIISNATYKEIGLLTCEATVNGHLYKTNYLTHRQTNTIIDVQISTPSPVTLCRGHTLVLNCTATTPANTRVQMTWSYPDEKNKNASVRRRIDQSNSHANIFYSVLTIDGMTNSDQGLYTCRVRSGPSFKSVNTSVHIYDCSGGGGSGGGGSGGGGSAESKYGPPCPPCPAPELLGGPSVFLFPPKPKDTLMISRTPEVTCVVVDVSHEDPEVKFNWYVDGVEVHNAKTKPREEQYNSTYRVVSVLTVLHQDWLNGKEYKCKVSNKALPAPIEKTISKAKGQPREPQVYTLPPSRDELTKNQVSLTCLVKGFYPSDIAVEWESNGQPENNYKTTPPVLDSDGSFFLYSKLTVDKSRWQQGNVFSCSVMHEALHNHYTQKSLSLSPG

SEQ ID NO: 9 - protein, 689 aa, synthetic construct
QVQLQESGPGLVKPSETLSITCTVSGFSLSNYDISWIRQPPGKGLEWLGVIWTGGATNYNPALKSRLTISRDNSKNQVSLKMSSVTAADTAVYYCVRDSNYRYDEPFTYWGQGTLVTVSSGGGGSGGGGSGGGGSGGGGSEIVLTQSPDTLSVTPKEKVTLTCRASQSIGTNIHWFQQKPGQSPKLLIKYASESISGVPSRFSGSGSGTDFTLTINSVEAEDAATYYCQQSNSWPYTFGQGTKLEIKRGGGGSGGGGSDTGRPFVEMYSEIPEIIHMTEGRELVIPCRVTSPNITVTLKKFPLDTLIPDGKRIIWDSRKGFIISNATYKEIGLLTCEATVNGHLYKTNYLTHRQTNTIIDVQISTPSPVTLCRGHTLVLNCTATTPANTRVQMTWSYPDEKNKNASVRRRIDQSNSHANIFYSVLTIDGMTNSDQGLYTCRVRSGPSFKSVNTSVHIYDCSSGDATPTSPPSPAPELLGGPSVFLFPPKPKDTLMISRTPEVTCVVVDVSHEDPEVKFNWYVDGVEVHNAKTKPREEQYNSTYRVVSVLTVLHQDWLNGKEYKCKVSNKALPAPIEKTISKAKGQPREPQVYTLPPSRDELTKNQVSLTCLVKGFYPSDIAVEWESNGQPENNYKTTPPVLDSDGSFFLYSKLTVDKSRWQQGNVFSCSVMHEALHNHYTQKSLSLSPG

SEQ ID NO: 10 - protein, 708 aa, synthetic construct
QVQLQESGPGLVKPSETLSITCTVSGFSLSNYDISWIRQPPGKGLEWLGVIWTGGATNYNPALKSRLTISRDNSKNQVSLKMSSVTAADTAVYYCVRDSNYRYDEPFTYWGQGTLVTVSSGGGGSGGGGSGGGGSGGGGSEIVLTQSPDTLSVTPKEKVTLTCRASQSIGTNIHWFQQKPGQSPKLLIKYASESISGVPSRFSGSGSGTDFTLTINSVEAEDAATYYCQQSNSWPYTFGQGTKLEIKRGSAEPKAGGGGSGGGGSGGGGSGRPFVEMYSEIPEIIHMTEGRELVIPCRVTSPNITVTLKKFPLDTLIPDGKRIIWDSRKGFIISNATYKEIGLLTCEATVNGHLYKTNYLTHRQTNTIIDVQISTPSPVTLCRGHTLVLNCTATTPANTRVQMTWSYPDEKNKNASVRRRIDQSNSHANIFYSVLTIDGMTNSDQGLYTCRVRSGPSFKSVNTSVHIYDCGSSGGSSGEPKSDATPTCPPCPAPELLGGPSVFLFPPKPKDTLMISRTPEVTCVVVDVSHEDPEVKFNWYVDGVEVHNAKTKPREEQYNSTYRVVSVLTVLHQDWLNGKEYKCKVSNKALPAPIEKTISKAKGQPREPQVYTLPPSRDELTKNQVSLTCLVKGFYPSDIAVEWESNGQPENNYKTTPPVLDSDGSFFLYSKLTVDKSRWQQGNVFSCSVMHEALHNHYTQKSLSLSPG

SEQ ID NO: 11 - protein, 708 aa, synthetic construct
QVQLQESGPGLVKPSETLSITCTVSGFSLSNYDISWIRQPPGKGLEWLGVIWTGGATNYNPALKSRLTISRDNSKNQVSLKMSSVTAADTAVYYCVRDSNYRYDEPFTYWGQGTLVTVSSGGGGSGGGGSGGGGSGGGGSEIVLTQSPDTLSVTPKEKVTLTCRASQSIGTNIHWFQQKPGQSPKLLIKYASESISGVPSRFSGSGSGTDFTLTINSVEAEDAATYYCQQSNSWPYTFGQGTKLEIKRGSGGGGSGGGGSGGGGSGGGGSGRPFVEMYSEIPEIIHMTEGRELVIPCRVTSPNITVTLKKFPLDTLIPDGKRIIWDSRKGFIISNATYKEIGLLTCEATVNGHLYKTNYLTHRQTNTIIDVQISTPSPVELCVGETLVLNCTATTPANTRVQMTWSYPDEKNKNASVRRRIDQSNSHANIFYSVLTIDGMTNSDKGLYTCRVRSGPSFKSVNTSVHIYDCGSSGGSSGEPKSDATPTCPPCPAPELLGGPSVFLFPPKPKDTLMISRTPEVTCVVVDVSHEDPEVKFNWYVDGVEVHNAKTKPREEQYNSTYRVVSVLTVLHQDWLNGKEYKCKVSNKALPAPIEKTISKAKGQPREPQVYTLPPSRDELTKNQVSLTCLVKGFYPSDIAVEWESNGQPENNYKTTPPVLDSDGSFFLYSKLTVDKSRWQQGNVFSCSVMHEALHNHYTQKSLSLSPG

SEQ ID NO: 12 - protein, 698 aa, synthetic construct
QVQLQESGPGLVKPSETLSITCTVSGFSLSNYDISWIRQPPGKGLEWLGVIWTGGATNYNPALKSRLTISRDNSKNQVSLKMSSVTAADTAVYYCVRDSNYRYDEPFTYWGQGTLVTVSSGGGGSGGGGSGGGGSGGGGSEIVLTQSPDTLSVTPKEKVTLTCRASQSIGTNIHWFQQKPGQSPKLLIKYASESISGVPSRFSGSGSGTDFTLTINSVEAEDAATYYCQQSNSWPYTFGQGTKLEIKRGGGGSGGGGSDTGRPFVEMYSEIPEIIHMTEGRELVIPCRVTSPNITVTLKKFPLDTLIPDGKRIIWDSRKGFIISNATYKEIGLLTCEATVNGHLYKTNYLTHRQTNTIIDVQISTPSPVELCVGETLVLNCTATTPANTRVQMTWSYPDEKNKNASVRRRIDQSNSHANIFYSVLTIDGMTNSDKGLYTCRVRSGPSFKSVNTSVHIYDCGSSGGSSGEPKSDATPTCPPCPAPELLGGPSVFLFPPKPKDTLMISRTPEVTCVVVDVSHEDPEVKFNWYVDGVEVHNAKTKPREEQYNSTYRVVSVLTVLHQDWLNGKEYKCKVSNKALPAPIEKTISKAKGQPREPQVYTLPPSRDELTKNQVSLTCLVKGFYPSDIAVEWESNGQPENNYKTTPPVLDSDGSFFLYSKLTVDKSRWQQGNVFSCSVMHEALHNHYTQKSLSLSPG

SEQ ID NO: 13 - protein, 720 aa, synthetic construct
  MUTAGEN 494: note = The residue of Serine was mutated to Cysteine
QVQLQESGPGLVKPSETLSITCTVSGFSLSNYDISWIRQPPGKGLEWLGVIWTGGATNYNPALKSRLTISRDNSKNQVSLKMSSVTAADTAVYYCVRDSNYRYDEPFTYWGQGTLVTVSSGGGGSGGGGSGGGGSGGGGSEIVLTQSPDTLSVTPKEKVTLTCRASQSIGTNIHWFQQKPGQSPKLLIKYASESISGVPSRFSGSGSGTDFTLTINSVEAEDAATYYCQQSNSWPYTFGQGTKLEIKRGSGGGGSGGGGSGGGGSGGGGSGRPFVEMYSEIPEIIHMTEGRELVIPCRVTSPNITVTLKKFPLDTLIPDGKRIIWDSRKGFIISNATYKEIGLLTCEATVNGHLYKTNYLTHRQTNTIIDVQISTPSPVELCVGETLVLNCTATTPANTRVQMTWSYPDEKNKNASVRRRIDQSNSHANIFYSVLTIDGMTNSDKGLYTCRVRSGPSFKSVNTSVHIYDCSNTGSGGEEKKKEKEKEEQEERSCDTPPTCPPCPAPELLGGPSVFLFPPKPKDTLMISRTPEVTCVVVDVSHEDPEVKFNWYVDGVEVHNAKTKPREEQYNSTYRVVSVLTVLHQDWLNGKEYKCKVSNKALPAPIEKTISKAKGQPREPQVYTLPPSRDELTKNQVSLTCLVKGFYPSDIAVEWESNGQPENNYKTTPPVLDSDGSFFLYSKLTVDKSRWQQGNVFSCSVMHEALHNHYTQKSLSLSPG

SEQ ID NO: 14 - protein, 715 aa, synthetic construct
QVQLQESGPGLVKPSETLSITCTVSGFSLSNYDISWIRQPPGKGLEWLGVIWTGGATNYNPALKSRLTISRDNSKNQVSLKMSSVTAADTAVYYCVRDSNYRYDEPFTYWGQGTLVTVSSGGGGSGGGGSGGGGSGGGGSEIVLTQSPDTLSVTPKEKVTLTCRASQSIGTNIHWFQQKPGQSPKLLIKYASESISGVPSRFSGSGSGTDFTLTINSVEAEDAATYYCQQSNSWPYTFGQGTKLEIKRGSGGGGSGGGGSGGGGSGGGGSGRPFVEMYSEIPEIIHMTEGRELVIPCRVTSPNITVTLKKFPLDTLIPDGKRIIWDSRKGFIISNATYKEIGLLTCEATVNGHLYKTNYLTHRQTNTIIDVQISTPSPVELCVGETLVLNCTATTPANTRVQMTWSYPDEKNKNASVRRRIDQSNSHANIFYSVLTIDGMTNSDKGLYTCRVRSGPSFKSVNTSVHIYDCSGGGGSGGGGSGGGGSAESKYGPPCPPCPAPELLGGPSVFLFPPKPKDTLMISRTPEVTCVVVDVSHEDPEVKFNWYVDGVEVHNAKTKPREEQYNSTYRVVSVLTVLHQDWLNGKEYKCKVSNKALPAPIEKTISKAKGQPREPQVYTLPPSRDELTKNQVSLTCLVKGFYPSDIAVEWESNGQPENNYKTTPPVLDSDGSFFLYSKLTVDKSRWQQGNVFSCSVMHEALHNHYTQKSLSLSPG

SEQ ID NO: 15 - protein, 689 aa, synthetic construct
QVQLQESGPGLVKPSETLSITCTVSGFSLSNYDISWIRQPPGKGLEWLGVIWTGGATNYNPALKSRLTISRDNSKNQVSLKMSSVTAADTAVYYCVRDSNYRYDEPFTYWGQGTLVTVSSGGGGSGGGGSGGGGSGGGGSEIVLTQSPDTLSVTPKEKVTLTCRASQSIGTNIHWFQQKPGQSPKLLIKYASESISGVPSRFSGSGSGTDFTLTINSVEAEDAATYYCQQSNSWPYTFGQGTKLEIKRGGGGSGGGGSDTGRPFVEMYSEIPEIIHMTEGRELVIPCRVTSPNITVTLKKFPLDTLIPDGKRIIWDSRKGFIISNATYKEIGLLTCEATVNGHLYKTNYLTHRQTNTIIDVQISTPSPVELCVGETLVLNCTATTPANTRVQMTWSYPDEKNKNASVRRRIDQSNSHANIFYSVLTIDGMTNSDKGLYTCRVRSGPSFKSVNTSVHIYDCSSGDATPTSPPSPAPELLGGPSVFLFPPKPKDTLMISRTPEVTCVVVDVSHEDPEVKFNWYVDGVEVHNAKTKPREEQYNSTYRVVSVLTVLHQDWLNGKEYKCKVSNKALPAPIEKTISKAKGQPREPQVYTLPPSRDELTKNQVSLTCLVKGFYPSDIAVEWESNGQPENNYKTTPPVLDSDGSFFLYSKLTVDKSRWQQGNVFSCSVMHEALHNHYTQKSLSLSPG

SEQ ID NO: 16 - protein, 708 aa, synthetic construct
QVQLQESGPGLVKPSETLSITCTVSGFSLSNYDISWIRQPPGKGLEWLGVIWTGGATNYNPALKSRLTISRDNSKNQVSLKMSSVTAADTAVYYCVRDSNYRYDEPFTYWGQGTLVTVSSGGGGSGGGGSGGGGSGGGGSEIVLTQSPDTLSVTPKEKVTLTCRASQSIGTNIHWFQQKPGQSPKLLIKYASESISGVPSRFSGSGSGTDFTLTINSVEAEDAATYYCQQSNSWPYTFGQGTKLEIKRGSAEPKAGGGGSGGGGSGGGGSGRPFVEMYSEIPEIIHMTEGRELVIPCRVTSPNITVTLKKFPLDTLIPDGKRIIWDSRKGFIISNATYKEIGLLTCEATVNGHLYKTNYLTHRQTNTIIDVQISTPSPVELCVGETLVLNCTATTPANTRVQMTWSYPDEKNKNASVRRRIDQSNSHANIFYSVLTIDGMTNSDKGLYTCRVRSGPSFKSVNTSVHIYDCGSSGGSSGEPKSDATPTCPPCPAPELLGGPSVFLFPPKPKDTLMISRTPEVTCVVVDVSHEDPEVKFNWYVDGVEVHNAKTKPREEQYNSTYRVVSVLTVLHQDWLNGKEYKCKVSNKALPAPIEKTISKAKGQPREPQVYTLPPSRDELTKNQVSLTCLVKGFYPSDIAVEWESNGQPENNYKTTPPVLDSDGSFFLYSKLTVDKSRWQQGNVFSCSVMHEALHNHYTQKSLSLSPG

SEQ ID NO: 17 - protein, 708 aa, synthetic construct
QVQLQESGPGLVKPSETLSITCTVSGFSLSNYDISWIRQPPGKGLEWLGVIWTGGATNYNPALKSRLTISRDNSKNQVSLKMSSVTAADTAVYYCVRDSNYRYDEPFTYWGQGTLVTVSSGGGGSGGGGSGGGGSGGGGSEIVLTQSPDTLSVTPKEKVTLTCRASQSIGTNIHWFQQKPGQSPKLLIKYASESISGVPSRFSGSGSGTDFTLTINSVEAEDAATYYCQQSNSWPYTFGQGTKLEIKRGSGGGGSGGGGSGGGGSGGGGSGRPFVEMYSEIPEIIHMTEGRELVIPCRVTSPNITVTLKKFPLDTLIPDGKRIIWDSRKGFIISNATYKEIGLLTCEATVNGHLYKTNYLTHRQTNTIIDVQISTPSPVELCVGETLVLNCTATTPDNTRVQMTWSYPDEKNKNASVRRRIDQSNSHANIFYSVLTIDGMTNSDKGLYTCRVRSGPSFKSVNTSVHIYDCGSSGGSSGEPKSDATPTCPPCPAPELLGGPSVFLFPPKPKDTLMISRTPEVTCVVVDVSHEDPEVKFNWYVDGVEVHNAKTKPREEQYNSTYRVVSVLTVLHQDWLNGKEYKCKVSNKALPAPIEKTISKAKGQPREPQVYTLPPSRDELTKNQVSLTCLVKGFYPSDIAVEWESNGQPENNYKTTPPVLDSDGSFFLYSKLTVDKSRWQQGNVFSCSVMHEALHNHYTQKSLSLSPG

SEQ ID NO: 18 - protein, 698 aa, synthetic construct
QVQLQESGPGLVKPSETLSITCTVSGFSLSNYDISWIRQPPGKGLEWLGVIWTGGATNYNPALKSRLTISRDNSKNQVSLKMSSVTAADTAVYYCVRDSNYRYDEPFTYWGQGTLVTVSSGGGGSGGGGSGGGGSGGGGSEIVLTQSPDTLSVTPKEKVTLTCRASQSIGTNIHWFQQKPGQSPKLLIKYASESISGVPSRFSGSGSGTDFTLTINSVEAEDAATYYCQQSNSWPYTFGQGTKLEIKRGGGGSGGGGSDTGRPFVEMYSEIPEIIHMTEGRELVIPCRVTSPNITVTLKKFPLDTLIPDGKRIIWDSRKGFIISNATYKEIGLLTCEATVNGHLYKTNYLTHRQTNTIIDVQISTPSPVELCVGETLVLNCTATTPDNTRVQMTWSYPDEKNKNASVRRRIDQSNSHANIFYSVLTIDGMTNSDKGLYTCRVRSGPSFKSVNTSVHIYDCGSSGGSSGEPKSDATPTCPPCPAPELLGGPSVFLFPPKPKDTLMISRTPEVTCVVVDVSHEDPEVKFNWYVDGVEVHNAKTKPREEQYNSTYRVVSVLTVLHQDWLNGKEYKCKVSNKALPAPIEKTISKAKGQPREPQVYTLPPSRDELTKNQVSLTCLVKGFYPSDIAVEWESNGQPENNYKTTPPVLDSDGSFFLYSKLTVDKSRWQQGNVFSCSVMHEALHNHYTQKSLSLSPG

SEQ ID NO: 19 - protein, 720 aa, synthetic construct
  MUTAGEN 493: note = The residue of Serine was mutated to Cysteine
QVQLQESGPGLVKPSETLSITCTVSGFSLSNYDISWIRQPPGKGLEWLGVIWTGGATNYNPALKSRLTISRDNSKNQVSLKMSSVTAADTAVYYCVRDSNYRYDEPFTYWGQGTLVTVSSGGGGSGGGGSGGGGSGGGGSEIVLTQSPDTLSVTPKEKVTLTCRASQSIGTNIHWFQQKPGQSPKLLIKYASESISGVPSRFSGSGSGTDFTLTINSVEAEDAATYYCQQSNSWPYTFGQGTKLEIKRGSGGGGSGGGGSGGGGSGGGGSGRPFVEMYSEIPEIIHMTEGRELVIPCRVTSPNITVTLKKFPLDTLIPDGKRIIWDSRKGFIISNATYKEIGLLTCEATVNGHLYKTNYLTHRQTNTIIDVQISTPSPVELCVGETLVLNCTATTPDNTRVQMTWSYPDEKNKNASVRRRIDQSNSHANIFYSVLTIDGMTNSDKGLYTCRVRSGPSFKSVNTSVHIYDCSNTGSGGEEKKKEKEKEEQEERSCDTPPTCPPCPAPELLGGPSVFLFPPKPKDTLMISRTPEVTCVVVDVSHEDPEVKFNWYVDGVEVHNAKTKPREEQYNSTYRVVSVLTVLHQDWLNGKEYKCKVSNKALPAPIEKTISKAKGQPREPQVYTLPPSRDELTKNQVSLTCLVKGFYPSDIAVEWESNGQPENNYKTTPPVLDSDGSFFLYSKLTVDKSRWQQGNVFSCSVMHEALHNHYTQKSLSLSPG

SEQ ID NO: 20 - protein, 715 aa, synthetic construct
QVQLQESGPGLVKPSETLSITCTVSGFSLSNYDISWIRQPPGKGLEWLGVIWTGGATNYNPALKSRLTISRDNSKNQVSLKMSSVTAADTAVYYCVRDSNYRYDEPFTYWGQGTLVTVSSGGGGSGGGGSGGGGSGGGGSEIVLTQSPDTLSVTPKEKVTLTCRASQSIGTNIHWFQQKPGQSPKLLIKYASESISGVPSRFSGSGSGTDFTLTINSVEAEDAATYYCQQSNSWPYTFGQGTKLEIKRGSGGGGSGGGGSGGGGSGGGGSGRPFVEMYSEIPEIIHMTEGRELVIPCRVTSPNITVTLKKFPLDTLIPDGKRIIWDSRKGFIISNATYKEIGLLTCEATVNGHLYKTNYLTHRQTNTIIDVQISTPSPVELCVGETLVLNCTATTPDNTRVQMTWSYPDEKNKNASVRRRIDQSNSHANIFYSVLTIDGMTNSDKGLYTCRVRSGPSFKSVNTSVHIYDCSGGGGSGGGGSGGGGSAESKYGPPCPPCPAPELLGGPSVFLFPPKPKDTLMISRTPEVTCVVVDVSHEDPEVKFNWYVDGVEVHNAKTKPREEQYNSTYRVVSVLTVLHQDWLNGKEYKCKVSNKALPAPIEKTISKAKGQPREPQVYTLPPSRDELTKNQVSLTCLVKGFYPSDIAVEWESNGQPENNYKTTPPVLDSDGSFFLYSKLTVDKSRWQQGNVFSCSVMHEALHNHYTQKSLSLSPG

SEQ ID NO: 21 - protein, 689 aa, synthetic construct
QVQLQESGPGLVKPSETLSITCTVSGFSLSNYDISWIRQPPGKGLEWLGVIWTGGATNYNPALKSRLTISRDNSKNQVSLKMSSVTAADTAVYYCVRDSNYRYDEPFTYWGQGTLVTVSSGGGGSGGGGSGGGGSGGGGSEIVLTQSPDTLSVTPKEKVTLTCRASQSIGTNIHWFQQKPGQSPKLLIKYASESISGVPSRFSGSGSGTDFTLTINSVEAEDAATYYCQQSNSWPYTFGQGTKLEIKRGGGGSGGGGSDTGRPFVEMYSEIPEIIHMTEGRELVIPCRVTSPNITVTLKKFPLDTLIPDGKRIIWDSRKGFIISNATYKEIGLLTCEATVNGHLYKTNYLTHRQTNTIIDVQISTPSPVELCVGETLVLNCTATTPDNTRVQMTWSYPDEKNKNASVRRRIDQSNSHANIFYSVLTIDGMTNSDKGLYTCRVRSGPSFKSVNTSVHIYDCSSGDATPTSPPSPAPELLGGPSVFLFPPKPKDTLMISRTPEVTCVVVDVSHEDPEVKFNWYVDGVEVHNAKTKPREEQYNSTYRVVSVLTVLHQDWLNGKEYKCKVSNKALPAPIEKTISKAKGQPREPQVYTLPPSRDELTKNQVSLTCLVKGFYPSDIAVEWESNGQPENNYKTTPPVLDSDGSFFLYSKLTVDKSRWQQGNVFSCSVMHEALHNHYTQKSLSLSPG

SEQ ID NO: 22 - protein, 708 aa, synthetic construct
QVQLQESGPGLVKPSETLSITCTVSGFSLSNYDISWIRQPPGKGLEWLGVIWTGGATNYNPALKSRLTISRDNSKNQVSLKMSSVTAADTAVYYCVRDSNYRYDEPFTYWGQGTLVTVSSGGGGSGGGGSGGGGSGGGGSEIVLTQSPDTLSVTPKEKVTLTCRASQSIGTNIHWFQQKPGQSPKLLIKYASESISGVPSRFSGSGSGTDFTLTINSVEAEDAATYYCQQSNSWPYTFGQGTKLEIKRGSAEPKAGGGGSGGGGSGGGGSGRPFVEMYSEIPEIIHMTEGRELVIPCRVTSPNITVTLKKFPLDTLIPDGKRIIWDSRKGFIISNATYKEIGLLTCEATVNGHLYKTNYLTHRQTNTIIDVQISTPSPVELCVGETLVLNCTATTPDNTRVQMTWSYPDEKNKNASVRRRIDQSNSHANIFYSVLTIDGMTNSDKGLYTCRVRSGPSFKSVNTSVHIYDCGSSGGSSGEPKSDATPTCPPCPAPELLGGPSVFLFPPKPKDTLMISRTPEVTCVVVDVSHEDPEVKFNWYVDGVEVHNAKTKPREEQYNSTYRVVSVLTVLHQDWLNGKEYKCKVSNKALPAPIEKTISKAKGQPREPQVYTLPPSRDELTKNQVSLTCLVKGFYPSDIAVEWESNGQPENNYKTTPPVLDSDGSFFLYSKLTVDKSRWQQGNVFSCSVMHEALHNHYTQKSLSLSPG

SEQ ID NO: 23 - protein, 720 aa, synthetic construct
QVQLQESGPGLVKPSETLSITCTVSGFSLSNYDISWIRQPPGKGLEWLGVIWTGGATNYNPALKSRLTISRDNSKNQVSLKMSSVTAADTAVYYCVRDSNYRYDEPFTYWGQGTLVTVSSGGGGSGGGGSGGGGSGGGGSEIVLTQSPDTLSVTPKEKVTLTCRASQSIGTNIHWFQQKPGQSPKLLIKYASESISGVPSRFSGSGSGTDFTLTINSVEAEDAATYYCQQSNSWPYTFGQGTKLEIKRGSAEPKAGGGGSGGGGSGGGGSGRPFVEMYSEIPEIIHMTEGRELVIPCRVTSPNITVTLKKFPLDTLIPDGKRIIWDSRKGFIISNATYKEIGLLTCEATVNGHLYKTNYLTHRQTNTIIDVQISTPSPVELCVGETLVLNCTATTPANTRVQMTWSYPDEKNKNASVRRRIDQSNSHANIFYSVLTIDGMTNSDKGLYTCRVRSGPSFKSVNTSVHIYDCSNTGSGGEEKKKEKEKEEQEERSSDTPPTCPPCPAPELLGGPSVFLFPPKPKDTLMISRTPEVTCVVVDVSHEDPEVKFNWYVDGVEVHNAKTKPREEQYNSTYRVVSVLTVLHQDWLNGKEYKCKVSNKALPAPIEKTISKAKGQPREPQVYTLPPSRDELTKNQVSLTCLVKGFYPSDIAVEWESNGQPENNYKTTPPVLDSDGSFFLYSKLTVDKSRWQQGNVFSCSVMHEALHNHYTQKSLSLSPG

SEQ ID NO: 24 - protein, 720 aa, synthetic construct
QVQLQESGPGLVKPSETLSITCTVSGFSLSNYDISWIRQPPGKGLEWLGVIWTGGATNYNPALKSRLTISRDNSKNQVSLKMSSVTAADTAVYYCVRDSNYRYDEPFTYWGQGTLVTVSSGGGGSGGGGSGGGGSGGGGSEIVLTQSPDTLSVTPKEKVTLTCRASQSIGTNIHWFQQKPGQSPKLLIKYASESISGVPSRFSGSGSGTDFTLTINSVEAEDAATYYCQQSNSWPYTFGQGTKLEIKRGSGGGGSGGGGSGGGGSGGGGSGRPFVEMYSEIPEIIHMTEGRELVIPCRVTSPNITVTLKKFPLDTLIPDGKRIIWDSRKGFIISNATYKEIGLLTCEATVNGHLYKTNYLTHRQTNTIIDVQISTPSPVELCVGETLVLNCTATTPANTRVQMTWSYPDEKNKNASVRRRIDQSNSHANIFYSVLTIDGMTNSDKGLYTCRVRSGPSFKSVNTSVHIYDCSNTGSGGEEKKKEKEKEEQEERSSDTPPTCPPCPAPELLGGPSVFLFPPKPKDTLMISRTPEVTCVVVDVSHEDPEVKFNWYVDGVEVHNAKTKPREEQYNSTYRVVSVLTVLHQDWLNGKEYKCKVSNKALPAPIEKTISKAKGQPREPQVYTLPPSRDELTKNQVSLTCLVKGFYPSDIAVEWESNGQPENNYKTTPPVLDSDGSFFLYSKLTVDKSRWQQGNVFSCSVMHEALHNHYTQKSLSLSPG

SEQ ID NO: 25 - protein, 715 aa, synthetic construct
QVQLQESGPGLVKPSETLSITCTVSGFSLSNYDISWIRQPPGKGLEWLGVIWTGGATNYNPALKSRLTISRDNSKNQVSLKMSSVTAADTAVYYCVRDSNYRYDEPFTYWGQGTLVTVSSGGGGSGGGGSGGGGSGGGGSEIVLTQSPDTLSVTPKEKVTLTCRASQSIGTNIHWFQQKPGQSPKLLIKYASESISGVPSRFSGSGSGTDFTLTINSVEAEDAATYYCQQSNSWPYTFGQGTKLEIKRGSAEPKAGGGGSGGGGSGGGGSGRPFVEMYSEIPEIIHMTEGRELVIPCRVTSPNITVTLKKFPLDTLIPDGKRIIWDSRKGFIISNATYKEIGLLTCEATVNGHLYKTNYLTHRQTNTIIDVQISTPSPVELCVGETLVLNCTATTPANTRVQMTWSYPDEKNKNASVRRRIDQSNSHANIFYSVLTIDGMTNSDKGLYTCRVRSGPSFKSVNTSVHIYDCSGGGGSGGGGSGGGGSAESKYGPPCPPCPAPEAAGGPSVFLFPPKPKDTLMISRTPEVTCVVVDVSQEDPEVQFNWYVDGVEVHNAKTKPREEQFNSTYRVVSVLTVLHQDWLNGKEYKCKVSNKGLPSSIEKTISKAKGQPREPQVYTLPPSQEEMTKNQVSLTCLVKGFYPSDIAVEWESNGQPENNYKTTPPVLDSDGSFFLYSRLTVDKSRWQEGNVFSCSVMHEALHNHYTQKSLSLSLG

SEQ ID NO: 26 - protein, 715 aa, synthetic construct
QVQLQESGPGLVKPSETLSITCTVSGFSLSNYDISWIRQPPGKGLEWLGVIWTGGATNYNPALKSRLTISRDNSKNQVSLKMSSVTAADTAVYYCVRDSNYRYDEPFTYWGQGTLVTVSSGGGGSGGGGSGGGGSGGGGSEIVLTQSPDTLSVTPKEKVTLTCRASQSIGTNIHWFQQKPGQSPKLLIKYASESISGVPSRFSGSGSGTDFTLTINSVEAEDAATYYCQQSNSWPYTFGQGTKLEIKRGSGGGGSGGGGSGGGGSGGGGSGRPFVEMYSEIPEIIHMTEGRELVIPCRVTSPNITVTLKKFPLDTLIPDGKRIIWDSRKGFIISNATYKEIGLLTCEATVNGHLYKTNYLTHRQTNTIIDVQISTPSPVELCVGETLVLNCTATTPANTRVQMTWSYPDEKNKNASVRRRIDQSNSHANIFYSVLTIDGMTNSDKGLYTCRVRSGPSFKSVNTSVHIYDCSGGGGSGGGGSGGGGSAESKYGPPCPPCPAPEAAGGPSVFLFPPKPKDTLMISRTPEVTCVVVDVSQEDPEVQFNWYVDGVEVHNAKTKPREEQFNSTYRVVSVLTVLHQDWLNGKEYKCKVSNKGLPSSIEKTISKAKGQPREPQVYTLPPSQEEMTKNQVSLTCLVKGFYPSDIAVEWESNGQPENNYKTTPPVLDSDGSFFLYSRLTVDKSRWQEGNVFSCSVMHEALHNHYTQKSLSLSLG

SEQ ID NO: 27 - protein, 720 aa, synthetic construct
QVQLQESGPGLVKPSETLSITCTVSGFSLSNYDISWIRQPPGKGLEWLGVIWTGGATNYNPALKSRLTISRDNSKNQVSLKMSSVTAADTAVYYCVRDSNYRYDEPFTYWGQGTLVTVSSGGGGSGGGGSGGGGSGGGGSEIVLTQSPDTLSVTPKEKVTLTCRASQSIGTNIHWFQQKPGQSPKLLIKYASESISGVPSRFSGSGSGTDFTLTINSVEAEDAATYYCQQSNSWPYTFGQGTKLEIKRGSAEPKAGGGGSGGGGSGGGGSGRPFVEMYSEIPEIIHMTEGRELVIPCRVTSPNITVTLKKFPLDTLIPDGKRIIWDSRKGFIISNATYKEIGLLTCEATVNGHLYKTNYLTHRQTNTIIDVQISTPSPVELCVGETLVLNCTATTPANTRVQMTWSYPDEKNKNASVRRRIDQSNSHANIFYSVLTIDGMTNSDKGLYTCRVRSGPSFKSVNTSVHIYDCSNTGSGGEEKKKEKEKEEQEERSSDTPPTCPPCPAPEAAGGPSVFLFPPKPKDTLMISRTPEVTCVVVDVSQEDPEVQFNWYVDGVEVHNAKTKPREEQFNSTYRVVSVLTVLHQDWLNGKEYKCKVSNKGLPSSIEKTISKAKGQPREPQVYTLPPSQEEMTKNQVSLTCLVKGFYPSDIAVEWESNGQPENNYKTTPPVLDSDGSFFLYSRLTVDKSRWQEGNVFSCSVMHEALHNHYTQKSLSLSLG

SEQ ID NO: 28 - protein, 720 aa, synthetic construct
QVQLQESGPGLVKPSETLSITCTVSGFSLSNYDISWIRQPPGKGLEWLGVIWTGGATNYNPALKSRLTISRDNSKNQVSLKMSSVTAADTAVYYCVRDSNYRYDEPFTYWGQGTLVTVSSGGGGSGGGGSGGGGSGGGGSEIVLTQSPDTLSVTPKEKVTLTCRASQSIGTNIHWFQQKPGQSPKLLIKYASESISGVPSRFSGSGSGTDFTLTINSVEAEDAATYYCQQSNSWPYTFGQGTKLEIKRGSGGGGSGGGGSGGGGSGGGGSGRPFVEMYSEIPEIIHMTEGRELVIPCRVTSPNITVTLKKFPLDTLIPDGKRIIWDSRKGFIISNATYKEIGLLTCEATVNGHLYKTNYLTHRQTNTIIDVQISTPSPVELCVGETLVLNCTATTPANTRVQMTWSYPDEKNKNASVRRRIDQSNSHANIFYSVLTIDGMTNSDKGLYTCRVRSGPSFKSVNTSVHIYDCSNTGSGGEEKKKEKEKEEQEERSSDTPPTCPPCPAPEAAGGPSVFLFPPKPKDTLMISRTPEVTCVVVDVSQEDPEVQFNWYVDGVEVHNAKTKPREEQFNSTYRVVSVLTVLHQDWLNGKEYKCKVSNKGLPSSIEKTISKAKGQPREPQVYTLPPSQEEMTKNQVSLTCLVKGFYPSDIAVEWESNGQPENNYKTTPPVLDSDGSFFLYSRLTVDKSRWQEGNVFSCSVMHEALHNHYTQKSLSLSLG

SEQ ID NO: 29 - protein, 720 aa, synthetic construct
QVQLQESGPGLVKPSETLSITCTVSGFSLSNYDISWIRQPPGKGLEWLGVIWTGGATNYNPALKSRLTISRDNSKNQVSLKMSSVTAADTAVYYCVRDSNYRYDEPFTYWGQGTLVTVSSGGGGSGGGGSGGGGSGGGGSEIVLTQSPDTLSVTPKEKVTLTCRASQSIGTNIHWFQQKPGQSPKLLIKYASESISGVPSRFSGSGSGTDFTLTINSVEAEDAATYYCQQSNSWPYTFGQGTKLEIKRGSAEPKAGGGGSGGGGSGGGGSGRPFVEMYSEIPEIIHMTEGRELVIPCRVTSPNITVTLKKFPLDTLIPDGKRIIWDSRKGFIISNATYKEIGLLTCEATVNGHLYKTNYLTHRQTNTIIDVQISTPSPVELCVGETLVLNCTATTPANTRVQMTWSYPDEKNKNASVRRRIDQSNSHANIFYSVLTIDGMTNSDKGLYTCRVRSGPSFKSVNTSVHIYDCSNTGSGGEEKKKEKEKEEQEERSSDTPPTCPPCPAPEAAGGPSVFLFPPKPKDQLMISRTPEVTCVVVDVSQEDPEVQFNWYVDGVEVHNAKTKPREEQFNSTYRVVSVLTVLHQDWLNGKEYKCKVSNKGLPSSIEKTISKAKGQPREPQVYTLPPSQEEMTKNQVSLTCLVKGFYPSDIAVEWESNGQPENNYKTTPPVLDSDGSFFLYSRLTVDKSRWQEGNVFSCSVLHEALHNHYTQKSLSLSLG

SEQ ID NO: 30 - protein, 720 aa, synthetic construct
QVQLQESGPGLVKPSETLSITCTVSGFSLSNYDISWIRQPPGKGLEWLGVIWTGGATNYNPALKSRLTISRDNSKNQVSLKMSSVTAADTAVYYCVRDSNYRYDEPFTYWGQGTLVTVSSGGGGSGGGGSGGGGSGGGGSEIVLTQSPDTLSVTPKEKVTLTCRASQSIGTNIHWFQQKPGQSPKLLIKYASESISGVPSRFSGSGSGTDFTLTINSVEAEDAATYYCQQSNSWPYTFGQGTKLEIKRGSGGGGSGGGGSGGGGSGGGGSGRPFVEMYSEIPEIIHMTEGRELVIPCRVTSPNITVTLKKFPLDTLIPDGKRIIWDSRKGFIISNATYKEIGLLTCEATVNGHLYKTNYLTHRQTNTIIDVQISTPSPVELCVGETLVLNCTATTPANTRVQMTWSYPDEKNKNASVRRRIDQSNSHANIFYSVLTIDGMTNSDKGLYTCRVRSGPSFKSVNTSVHIYDCSNTGSGGEEKKKEKEKEEQEERSSDTPPTCPPCPAPEAAGGPSVFLFPPKPKDQLMISRTPEVTCVVVDVSQEDPEVQFNWYVDGVEVHNAKTKPREEQFNSTYRVVSVLTVLHQDWLNGKEYKCKVSNKGLPSSIEKTISKAKGQPREPQVYTLPPSQEEMTKNQVSLTCLVKGFYPSDIAVEWESNGQPENNYKTTPPVLDSDGSFFLYSRLTVDKSRWQEGNVFSCSVLHEALHNHYTQKSLSLSLG

SEQ ID NO: 31 - protein, 718 aa, synthetic construct
EVQLVESGGGLVQPGGSLRLSCAASGFTFSDSWIHWVRQAPGKGLEWVAWISPYGGSTYYADSVKGRFTISADTSKNTAYLQMNSLRAEDTAVYYCARRHWPGGFDYWGQGTLVTVSSGGGGSGGGGSGGGGSGGGGSDIQMTQSPSSLSASVGDRVTITCRASQDVSTAVAWYQQKPGKAPKLLIYSASFLYSGVPSRFSGSGSGTDFTLTISSLQPEDFATYYCQQYLYHPATFGQGTKVEIKRGSAEPKAGGGGSGGGGSGGGGSGRPFVEMYSEIPEIIHMTEGRELVIPCRVTSPNITVTLKKFPLDTLIPDGKRIIWDSRKGFIISNATYKEIGLLTCEATVNGHLYKTNYLTHRQTNTIIDVQISTPSPVELCVGETLVLNCTATTPANTRVQMTWSYPDEKNKNASVRRRIDQSNSHANIFYSVLTIDGMTNSDKGLYTCRVRSGPSFKSVNTSVHIYDCSNTGSGGEEKKKEKEKEEQEERSSDTPPTCPPCPAPELLGGPSVFLFPPKPKDTLMISRTPEVTCVVVDVSHEDPEVKFNWYVDGVEVHNAKTKPREEQYNSTYRVVSVLTVLHQDWLNGKEYKCKVSNKALPAPIEKTISKAKGQPREPQVYTLPPSRDELTKNQVSLTCLVKGFYPSDIAVEWESNGQPENNYKTTPPVLDSDGSFFLYSKLTVDKSRWQQGNVFSCSVMHEALHNHYTQKSLSLSPG

SEQ ID NO: 32 - protein, 718 aa, synthetic construct
EVQLVESGGGLVQPGGSLRLSCAASGFTFSDSWIHWVRQAPGKGLEWVAWISPYGGSTYYADSVKGRFTISADTSKNTAYLQMNSLRAEDTAVYYCARRHWPGGFDYWGQGTLVTVSSGGGGSGGGGSGGGGSGGGGSDIQMTQSPSSLSASVGDRVTITCRASQDVSTAVAWYQQKPGKAPKLLIYSASFLYSGVPSRFSGSGSGTDFTLTISSLQPEDFATYYCQQYLYHPATFGQGTKVEIKRGSGGGGSGGGGSGGGGSGGGGSGRPFVEMYSEIPEIIHMTEGRELVIPCRVTSPNITVTLKKFPLDTLIPDGKRIIWDSRKGFIISNATYKEIGLLTCEATVNGHLYKTNYLTHRQTNTIIDVQISTPSPVELCVGETLVLNCTATTPANTRVQMTWSYPDEKNKNASVRRRIDQSNSHANIFYSVLTIDGMTNSDKGLYTCRVRSGPSFKSVNTSVHIYDCSNTGSGGEEKKKEKEKEEQEERSSDTPPTCPPCPAPELLGGPSVFLFPPKPKDTLMISRTPEVTCVVVDVSHEDPEVKFNWYVDGVEVHNAKTKPREEQYNSTYRVVSVLTVLHQDWLNGKEYKCKVSNKALPAPIEKTISKAKGQPREPQVYTLPPSRDELTKNQVSLTCLVKGFYPSDIAVEWESNGQPENNYKTTPPVLDSDGSFFLYSKLTVDKSRWQQGNVFSCSVMHEALHNHYTQKSLSLSPG

SEQ ID NO: 33 - protein, 713 aa, synthetic construct
EVQLVESGGGLVQPGGSLRLSCAASGFTFSDSWIHWVRQAPGKGLEWVAWISPYGGSTYYADSVKGRFTISADTSKNTAYLQMNSLRAEDTAVYYCARRHWPGGFDYWGQGTLVTVSSGGGGSGGGGSGGGGSGGGGSDIQMTQSPSSLSASVGDRVTITCRASQDVSTAVAWYQQKPGKAPKLLIYSASFLYSGVPSRFSGSGSGTDFTLTISSLQPEDFATYYCQQYLYHPATFGQGTKVEIKRGSAEPKAGGGGSGGGGSGGGGSGRPFVEMYSEIPEIIHMTEGRELVIPCRVTSPNITVTLKKFPLDTLIPDGKRIIWDSRKGFIISNATYKEIGLLTCEATVNGHLYKTNYLTHRQTNTIIDVQISTPSPVELCVGETLVLNCTATTPANTRVQMTWSYPDEKNKNASVRRRIDQSNSHANIFYSVLTIDGMTNSDKGLYTCRVRSGPSFKSVNTSVHIYDCSGGGGSGGGGSGGGGSAESKYGPPCPPCPAPEAAGGPSVFLFPPKPKDQLMISRTPEVTCVVVDVSQEDPEVQFNWYVDGVEVHNAKTKPREEQFNSTYRVVSVLTVLHQDWLNGKEYKCKVSNKGLPSSIEKTISKAKGQPREPQVYTLPPSQEEMTKNQVSLTCLVKGFYPSDIAVEWESNGQPENNYKTTPPVLDSDGSFFLYSRLTVDKSRWQEGNVFSCSVLHEALHNHYTQKSLSLSLG

SEQ ID NO: 34 - protein, 713 aa, synthetic construct
EVQLVESGGGLVQPGGSLRLSCAASGFTFSDSWIHWVRQAPGKGLEWVAWISPYGGSTYYADSVKGRFTISADTSKNTAYLQMNSLRAEDTAVYYCARRHWPGGFDYWGQGTLVTVSSGGGGSGGGGSGGGGSGGGGSDIQMTQSPSSLSASVGDRVTITCRASQDVSTAVAWYQQKPGKAPKLLIYSASFLYSGVPSRFSGSGSGTDFTLTISSLQPEDFATYYCQQYLYHPATFGQGTKVEIKRGSGGGGSGGGGSGGGGSGGGGSGRPFVEMYSEIPEIIHMTEGRELVIPCRVTSPNITVTLKKFPLDTLIPDGKRIIWDSRKGFIISNATYKEIGLLTCEATVNGHLYKTNYLTHRQTNTIIDVQISTPSPVELCVGETLVLNCTATTPANTRVQMTWSYPDEKNKNASVRRRIDQSNSHANIFYSVLTIDGMTNSDKGLYTCRVRSGPSFKSVNTSVHIYDCSGGGGSGGGGSGGGGSAESKYGPPCPPCPAPEAAGGPSVFLFPPKPKDQLMISRTPEVTCVVVDVSQEDPEVQFNWYVDGVEVHNAKTKPREEQFNSTYRVVSVLTVLHQDWLNGKEYKCKVSNKGLPSSIEKTISKAKGQPREPQVYTLPPSQEEMTKNQVSLTCLVKGFYPSDIAVEWESNGQPENNYKTTPPVLDSDGSFFLYSRLTVDKSRWQEGNVFSCSVLHEALHNHYTQKSLSLSLG

SEQ ID NO: 35 - protein, 718 aa, synthetic construct
EVQLVESGGGLVQPGGSLRLSCAASGFTFSDSWIHWVRQAPGKGLEWVAWISPYGGSTYYADSVKGRFTISADTSKNTAYLQMNSLRAEDTAVYYCARRHWPGGFDYWGQGTLVTVSSGGGGSGGGGSGGGGSGGGGSDIQMTQSPSSLSASVGDRVTITCRASQDVSTAVAWYQQKPGKAPKLLIYSASFLYSGVPSRFSGSGSGTDFTLTISSLQPEDFATYYCQQYLYHPATFGQGTKVEIKRGSAEPKAGGGGSGGGGSGGGGSGRPFVEMYSEIPEIIHMTEGRELVIPCRVTSPNITVTLKKFPLDTLIPDGKRIIWDSRKGFIISNATYKEIGLLTCEATVNGHLYKTNYLTHRQTNTIIDVQISTPSPVELCVGETLVLNCTATTPANTRVQMTWSYPDEKNKNASVRRRIDQSNSHANIFYSVLTIDGMTNSDKGLYTCRVRSGPSFKSVNTSVHIYDCSNTGSGGEEKKKEKEKEEQEERSSDTPPTCPPCPAPEAAGGPSVFLFPPKPKDQLMISRTPEVTCVVVDVSQEDPEVQFNWYVDGVEVHNAKTKPREEQFNSTYRVVSVLTVLHQDWLNGKEYKCKVSNKGLPSSIEKTISKAKGQPREPQVYTLPPSQEEMTKNQVSLTCLVKGFYPSDIAVEWESNGQPENNYKTTPPVLDSDGSFFLYSRLTVDKSRWQEGNVFSCSVLHEALHNHYTQKSLSLSLG

SEQ ID NO: 36 - protein, 718 aa, synthetic construct
EVQLVESGGGLVQPGGSLRLSCAASGFTFSDSWIHWVRQAPGKGLEWVAWISPYGGSTYYADSVKGRFTISADTSKNTAYLQMNSLRAEDTAVYYCARRHWPGGFDYWGQGTLVTVSSGGGGSGGGGSGGGGSGGGGSDIQMTQSPSSLSASVGDRVTITCRASQDVSTAVAWYQQKPGKAPKLLIYSASFLYSGVPSRFSGSGSGTDFTLTISSLQPEDFATYYCQQYLYHPATFGQGTKVEIKRGSGGGGSGGGGSGGGGSGGGGSGRPFVEMYSEIPEIIHMTEGRELVIPCRVTSPNITVTLKKFPLDTLIPDGKRIIWDSRKGFIISNATYKEIGLLTCEATVNGHLYKTNYLTHRQTNTIIDVQISTPSPVELCVGETLVLNCTATTPANTRVQMTWSYPDEKNKNASVRRRIDQSNSHANIFYSVLTIDGMTNSDKGLYTCRVRSGPSFKSVNTSVHIYDCSNTGSGGEEKKKEKEKEEQEERSSDTPPTCPPCPAPEAAGGPSVFLFPPKPKDQLMISRTPEVTCVVVDVSQEDPEVQFNWYVDGVEVHNAKTKPREEQFNSTYRVVSVLTVLHQDWLNGKEYKCKVSNKGLPSSIEKTISKAKGQPREPQVYTLPPSQEEMTKNQVSLTCLVKGFYPSDIAVEWESNGQPENNYKTTPPVLDSDGSFFLYSRLTVDKSRWQEGNVFSCSVLHEALHNHYTQKSLSLSLG

SEQ ID NO: 37 - protein, 497 aa, synthetic construct; identical to SEQ ID NO: 3

SEQ ID NO: 38 - protein, 467 aa, synthetic construct
EVQLVESGGGLVQPGGSLRLSCAASGFTFSDSWIHWVRQAPGKGLEWVAWISPYGGSTYYADSVKGRFTISADTSKNTAYLQMNSLRAEDTAVYYCARRHWPGGFDYWGQGTLVTVSSGGGGSGGGGSGGGGSGGGGSDIQMTQSPSSLSASVGDRVTITCRASQDVSTAVAWYQQKPGKAPKLLIYSASFLYSGVPSRFSGSGSGTDFTLTISSLQPEDFATYYCQQYLYHPATFGQGTKVEIKRCPPCPAPELLGGPSVFLFPPKPKDTLMISRTPEVTCVVVDVSHEDPEVKFNWYVDGVEVHNAKTKPREEQYNSTYRVVSVLTVLHQDWLNGKEYKCKVSNKALPAPIEKTISKAKGQPREPQVYTLPPSRDELTKNQVSLTCLVKGFYPSDIAVEWESNGQPENNYKTTPPVLDSDGSFFLYSKLTVDKSRWQQGNVFSCSVMHEALHNHYTQKSLSLSPG

SEQ ID NO: 39 - protein, 244 aa, synthetic construct
EVQLVESGGGLVQPGGSLRLSCAASGFTFSDSWIHWVRQAPGKGLEWVAWISPYGGSTYYADSVKGRFTISADTSKNTAYLQMNSLRAEDTAVYYCARRHWPGGFDYWGQGTLVTVSSGGGGSGGGGSGGGGSGGGGSDIQMTQSPSSLSASVGDRVTITCRASQDVSTAVAWYQQKPGKAPKLLIYSASFLYSGVPSRFSGSGSGTDFTLTISSLQPEDFATYYCQQYLYHPATFGQGTKVEI

SEQ ID NO: 40 - protein, 248 aa, synthetic construct
QVQLQESGPGLVKPSETLSITCTVSGFSLSNYDISWIRQPPGKGLEWLGVIWTGGATNYNPALKSRLTISRDNSKNQVSLKMSSVTAADTAVYYCVRDSNYRYDEPFTYWGQGTLVTVSSGGGGSGGGGSGGGGSGGGGSEIVLTQSPDTLSVTPKEKVTLTCRASQSIGTNIHWFQQKPGQSPKLLIKYASESISGVPSRFSGSGSGTDFTLTINSVEAEDAATYYCQQSNSWPYTFGQGTKLEIKR

SEQ ID NO: 41 - protein, 1338 aa, Homo sapiens
MVSYWDTGVLLCALLSCLLLTGSSSGSKLKDPELSLKGTQHIMQAGQTLHLQCRGEAAHKWSLPEMVSKESERLSITKSACGRNGKQFCSTLTLNTAQANHTGFYSCKYLAVPTSKKKETESAIYIFISDTGRPFVEMYSEIPEIIHMTEGRELVIPCRVTSPNITVTLKKFPLDTLIPDGKRIIWDSRKGFIISNATYKEIGLLTCEATVNGHLYKTNYLTHRQTNTIIDVQISTPRPVKLLRGHTLVLNCTATTPLNTRVQMTWSYPDEKNKRASVRRRIDQSNSHANIFYSVLTIDKMQNKDKGLYTCRVRSGPSFKSVNTSVHIYDKAFITVKHRKQQVLETVAGKRSYRLSMKVKAFPSPEVVWLKDGLPATEKSARYLTRGYSLIIKDVTEEDAGNYTILLSIKQSNVFKNLTATLIVNVKPQIYEKAVSSFPDPALYPLGSRQILTCTAYGIPQPTIKWFWHPCNHNHSEARCDFCSNNEESFILDADSNMGNRIESITQRMAIIEGKNKMASTLVVADSRISGIYICIASNKVGTVGRNISFYITDVPNGFHVNLEKMPTEGEDLKLSCTVNKFLYRDVTWILLRTVNNRTMHYSISKQKMAITKEHSITLNLTIMNVSLQDSGTYACRARNVYTGEEILQKKEITIRDQEAPYLLRNLSDHTVAISSSTTLDCHANGVPEPQITWFKNNHKIQQEPGIILGPGSSTLFIERVTEEDEGVYHCKATNQKGSVESSAYLTVQGTSDKSNLELITLTCTCVAATLFWLLLTLFIRKMKRSSSEIKTDYLSIIMDPDEVPLDEQCERLPYDASKWEFARERLKLGKSLGRGAFGKVVQASAFGIKKSPTCRTVAVKMLKEGATASEYKALMTELKILTHIGHHLNVVNLLGACTKQGGPLMVIVEYCKYGNLSNYLKSKRDLFFLNKDAALHMEPKKEKMEPGLEQGKKPRLDSVTSSESFASSGFQEDKSLSDVEEEEDSDGFYKEPITMEDLISYSFQVARGMEFLSSRKCIHRDLAARNILLSENNVVKICDFGLARDIYKNPDYVRKGDTRLPLKWMAPESIFDKIYSTKSDVWSYGVLLWEIFSLGGSPYPGVQMDEDFCSRLREGMRMRAPEYSTPEIYQIMLDCWHRDPKERPRFAELVEKLGDLLQANVQQDGKDYIPINAILTGNSGFTYSTPAFSEDFFKESISAPKFNSGSSDDVRYVNAFKFMSLERIKTFEELLPNATSMFDDYQGDSSTLLASPMLKRFTWTDSKPKASLKIDLRVTSKSKESGLSDVSRPSFCHSSCGHVSEGKRRFTYDHAELERKIACCSPPPDYNSVVLYSTPPI

SEQ ID NO: 42 - protein, 432 aa, synthetic construct
EFGRPFVEMYSEIPEIIHMTEGRELVIPCRVTSPNITVTLKKFPLDTLIPDGKRIIWDSRKGFIISNATYKEIGLLTCEATVNGHLYKTNYLTHRQTNTIIDVQISTPSPVTLLRGHTLVLNCTATTPLNTRVQMTWSYPDEKNKRASVRRRIDQSNSHANIFYSVLTIDKMQNKDKGLYTCRVRSGPSFKSVNTSVHIYDKALEDKTHTCPPCPAPELLGGPSVFLFPPKPKDTLMISRTPEVTCVVVDVSHEDPEVKFNWYVDGVEVHNAKTKPREEQYNSTYRVVSVLTVLHQDWLNGKEYKCKVSNKALPAPIEKTISKAKGQPREPQVYTLPPSREEMTKNQVSLTCLVKGFYPSDIAVEWESNGQPENNYKTTPPVLDSDGSFFLYSKLTVDKSRWQQGNVFSCSVMHEALHNHYTQKSLSLSPGK

SEQ ID NO: 43 - protein, 432 aa, synthetic construct
EFGRPFVEMYSEIPEIIHMTEGRELVIPCRVTSPNITVTLKKFPLDTLIPDGKRIIWDSRKGFIISNATYKEIGLLTCEATVNGHLYKTNYLTHRQTNTIIDVQISTPSPVTLLRGHTLVLNCTATTPLNTRVQMTWSYPDEKNKNASVRRRIDQSNSHANIFYSVLTIDKMQNKDKGLYTCRVRSGPSFKSVNTSVHIYDKALEDKTHTCPPCPAPELLGGPSVFLFPPKPKDTLMISRTPEVTCVVVDVSHEDPEVKFNWYVDGVEVHNAKTKPREEQYNSTYRVVSVLTVLHQDWLNGKEYKCKVSNKALPAPIEKTISKAKGQPREPQVYTLPPSREEMTKNQVSLTCLVKGFYPSDIAVEWESNGQPENNYKTTPPVLDSDGSFFLYSKLTVDKSRWQQGNVFSCSVMHEALHNHYTQKSLSLSPGK

SEQ ID NO: 44 - protein, 431 aa, synthetic construct
EFGRPFVEMYSEIPEIIHMTEGRELVIPCRVTSPNITVTLKKFPLDTLIPDGKRIIWDSRKGFIISNATYKEIGLLTCEATVNGHLYKTNYLTHRQTNTIIDVQISTPSPVELCVGETLVLNCTATTPANTRVQMTWSYPDEKNKNASVRRRIDQSNSHANIFYSVLTIDGMTNSDKGLYTCRVRSGPSFKSVNTSVHIYDCSSGDATPTSPPSPAPELLGGPSVFLFPPKPKDTLMISRTPEVTCVVVDVSHEDPEVKFNWYVDGVEVHNAKTKPREEQYNSTYRVVSVLTVLHQDWLNGKEYKCKVSNKALPAPIEKTISKAKGQPREPQVYTLPPSRDELTKNQVSLTCLVKGFYPSDIAVEWESNGQPENNYKTTPPVLDSDGSFFLYSKLTVDKSRWQQGNVFSCSVMHEALHNHYTQKSLSLSPG

SEQ ID NO: 45 - protein, 440 aa, synthetic construct
EFGRPFVEMYSEIPEIIHMTEGRELVIPCRVTSPNITVTLKKFPLDTLIPDGKRIIWDSRKGFIISNATYKEIGLLTCEATVNGHLYKTNYLTHRQTNTIIDVQISTPSPVELCVGETLVLNCTATTPANTRVQMTWSYPDEKNKNASVRRRIDQSNSHANIFYSVLTIDGMTNSDKGLYTCRVRSGPSFKSVNTSVHIYDCSKVDKKVEPKSSDTPPTCPPCPAPELLGGPSVFLFPPKPKDTLMISRTPEVTCVVVDVSHEDPEVKFNWYVDGVEVHNAKTKPREEQYNSTYRVVSVLTVLHQDWLNGKEYKCKVSNKALPAPIEKTISKAKGQPREPQVYTLPPSRDELTKNQVSLTCLVKGFYPSDIAVEWESNGQPENNYKTTPPVLDSDGSFFLYSKLTVDKSRWQQGNVFSCSVMHEALHNHYTQKSLSLSPG

SEQ ID NO: 46 - protein, 444 aa, synthetic construct
EFGRPFVEMYSEIPEIIHMTEGRELVIPCRVTSPNITVTLKKFPLDTLIPDGKRIIWDSRKGFIISNATYKEIGLLTCEATVNGHLYKTNYLTHRQTNTIIDVQISTPSPVELCVGETLVLNCTATTPANTRVQMTWSYPDEKNKNASVRRRIDQSNSHANIFYSVLTIDGMTNSDKGLYTCRVRSGPSFKSVNTSVHIYDCSGGGGSAEPKAGDATPPTCPPCPPCPAPELLGGPSVFLFPPKPKDTLMISRTPEVTCVVVDVSHEDPEVKFNWYVDGVEVHNAKTKPREEQYNSTYRVVSVLTVLHQDWLNGKEYKCKVSNKALPAPIEKTISKAKGQPREPQVYTLPPSRDELTKNQVSLTCLVKGFYPSDIAVEWESNGQPENNYKTTPPVLDSDGSFFLYSKLTVDKSRWQQGNVFSCSVMHEALHNHYTQKSLSLSPG

SEQ ID NO: 47 - protein, 447 aa, synthetic construct
EFGRPFVEMYSEIPEIIHMTEGRELVIPCRVTSPNITVTLKKFPLDTLIPDGKRIIWDSRKGFIISNATYKEIGLLTCEATVNGHLYKTNYLTHRQTNTIIDVQISTPSPVELCVGETLVLNCTATTPANTRVQMTWSYPDEKNKNASVRRRIDQSNSHANIFYSVLTIDGMTNSDKGLYTCRVRSGPSFKSVNTSVHIYDCSGGGGSGGGGSGGGGSAESKYGPPCPPCPAPELLGGPSVFLFPPKPKDTLMISRTPEVTCVVVDVSHEDPEVKFNWYVDGVEVHNAKTKPREEQYNSTYRVVSVLTVLHQDWLNGKEYKCKVSNKALPAPIEKTISKAKGQPREPQVYTLPPSRDELTKNQVSLTCLVKGFYPSDIAVEWESNGQPENNYKTTPPVLDSDGSFFLYSKLTVDKSRWQQGNVFSCSVMHEALHNHYTQKSLSLSPG

SEQ ID NO: 48 - protein, 452 aa, synthetic construct
EFGRPFVEMYSEIPEIIHMTEGRELVIPCRVTSPNITVTLKKFPLDTLIPDGKRIIWDSRKGFIISNATYKEIGLLTCEATVNGHLYKTNYLTHRQTNTIIDVQISTPSPVELCVGETLVLNCTATTPANTRVQMTWSYPDEKNKNASVRRRIDQSNSHANIFYSVLTIDGMTNSDKGLYTCRVRSGPSFKSVNTSVHIYDCSNTGSGGEEKKKEKEKEEQEERSSDTPPTCPPCPAPELLGGPSVFLFPPKPKDTLMISRTPEVTCVVVDVSHEDPEVKFNWYVDGVEVHNAKTKPREEQYNSTYRVVSVLTVLHQDWLNGKEYKCKVSNKALPAPIEKTISKAKGQPREPQVYTLPPSRDELTKNQVSLTCLVKGFYPSDIAVEWESNGQPENNYKTTPPVLDSDGSFFLYSKLTVDKSRWQQGNVFSCSVMHEALHNHYTQKSLSLSPG

SEQ ID NO: 49 - protein, 440 aa, synthetic construct
EFGRPFVEMYSEIPEIIHMTEGRELVIPCRVTSPNITVTLKKFPLDTLIPDGKRIIWDSRKGFIISNATYKEIGLLTCEATVNGHLYKTNYLTHRQTNTIIDVQISTPSPVELCVGETLVLNCTATTPANTRVQMTWSYPDEKNKNASVRRRIDQSNSHANIFYSVLTIDGMTNSDKGLYTCRVRSGPSFKSVNTSVHIYDCGSSGGSSGEPKSDATPTCPPCPAPELLGGPSVFLFPPKPKDTLMISRTPEVTCVVVDVSHEDPEVKFNWYVDGVEVHNAKTKPREEQYNSTYRVVSVLTVLHQDWLNGKEYKCKVSNKALPAPIEKTISKAKGQPREPQVYTLPPSRDELTKNQVSLTCLVKGFYPSDIAVEWESNGQPENNYKTTPPVLDSDGSFFLYSKLTVDKSRWQQGNVFSCSVMHEALHNHYTQKSLSLSPG

SEQ ID NO: 50 - protein, 440 aa, synthetic construct
EFGRPFVEMYSEIPEIIHMTEGRELVIPCRVTSPNITVTLKKFPLDTLIPDGKRIIWDSRKGFIISNATYKEIGLLTCEATVNGHLYKTNYLTHRQTNTIIDVQISTPSPVELCVGETLVLNCTATTPANTRVQMTWSYPDEKNKNASVRRRIDQSNSHANIFYSVLTIDGMTNSDKGLYTCRVRSGPSFKSVNTSVHIYDCSKVDKKVEPKSSDKTYTCPPCPAPELLGGPSVFLFPPKPKDTLMISRTPEVTCVVVDVSHEDPEVKFNWYVDGVEVHNAKTKPREEQYNSTYRVVSVLTVLHQDWLNGKEYKCKVSNKALPAPIEKTISKAKGQPREPQVYTLPPSRDELTKNQVSLTCLVKGFYPSDIAVEWESNGQPENNYKTTPPVLDSDGSFFLYSKLTVDKSRWQQGNVFSCSVMHEALHNHYTQKSLSLSPG

SEQ ID NO: 51 - protein, 440 aa, synthetic construct
EFGRPFVEMYSEIPEIIHMTEGRELVIPCRVTSPNITVTLKKFPLDTLIPDGKRIIWDSRKGFIISNATYKEIGLLTCEATVNGHLYKTNYLTHRQTNTIIDVQISTPSPVELCVGETLVLNCTATTPSNTRVQMTWSYPDEKNKNASVRRRIDQSNSHANIFYSVLTIDGMTNSDKGLYTCRVRSGPSFKSVNTSVHIYDCSKVDKKVEPKSSDTPPTCPPCPAPELLGGPSVFLFPPKPKDTLMISRTPEVTCVVVDVSHEDPEVKFNWYVDGVEVHNAKTKPREEQYNSTYRVVSVLTVLHQDWLNGKEYKCKVSNKALPAPIEKTISKAKGQPREPQVYTLPPSRDELTKNQVSLTCLVKGFYPSDIAVEWESNGQPENNYKTTPPVLDSDGSFFLYSKLTVDKSRWQQGNVFSCSVMHEALHNHYTQKSLSLSPG

SEQ ID NO: 52 - protein, 440 aa, synthetic construct
EFGRPFVEMYSEIPEIIHMTEGRELVIPCRVTSPNITVTLKKFPLDTLIPDGKRIIWDSRKGFIISNATYKEIGLLTCEATVNGHLYKTNYLTHRQTNTIIDVQISTPSPVELCVGETLVLNCTATTPDNTRVQMTWSYPDEKNKNASVRRRIDQSNSHANIFYSVLTIDGMTNSDKGLYTCRVRSGPSFKSVNTSVHIYDCSKVDKKVEPKSSDTPPTCPPCPAPELLGGPSVFLFPPKPKDTLMISRTPEVTCVVVDVSHEDPEVKFNWYVDGVEVHNAKTKPREEQYNSTYRVVSVLTVLHQDWLNGKEYKCKVSNKALPAPIEKTISKAKGQPREPQVYTLPPSRDELTKNQVSLTCLVKGFYPSDIAVEWESNGQPENNYKTTPPVLDSDGSFFLYSKLTVDKSRWQQGNVFSCSVMHEALHNHYTQKSLSLSPG

SEQ ID NO: 53 - protein, 447 aa, synthetic construct
EFGRPFVEMYSEIPEIIHMTEGRELVIPCRVTSPNITVTLKKFPLDTLIPDGKRIIWDSRKGFIISNATYKEIGLLTCEATVNGHLYKTNYLTHRQTNTIIDVQISTPSPVELCVGETLVLNCTATTPSNTRVQMTWSYPDEKNKNASVRRRIDQSNSHANIFYSVLTIDGMTNSDKGLYTCRVRSGPSFKSVNTSVHIYDCSGGGGSGGGGSGGGGSAESKYGPPCPPCPAPELLGGPSVFLFPPKPKDTLMISRTPEVTCVVVDVSHEDPEVKFNWYVDGVEVHNAKTKPREEQYNSTYRVVSVLTVLHQDWLNGKEYKCKVSNKALPAPIEKTISKAKGQPREPQVYTLPPSRDELTKNQVSLTCLVKGFYPSDIAVEWESNGQPENNYKTTPPVLDSDGSFFLYSKLTVDKSRWQQGNVFSCSVMHEALHNHYTQKSLSLSPG

SEQ ID NO: 54 - protein, 447 aa, synthetic construct
EFGRPFVEMYSEIPEIIHMTEGRELVIPCRVTSPNITVTLKKFPLDTLIPDGKRIIWDSRKGFIISNATYKEIGLLTCEATVNGHLYKTNYLTHRQTNTIIDVQISTPSPVELCVGETLVLNCTATTPDNTRVQMTWSYPDEKNKNASVRRRIDQSNSHANIFYSVLTIDGMTNSDKGLYTCRVRSGPSFKSVNTSVHIYDCSGGGGSGGGGSGGGGSAESKYGPPCPPCPAPELLGGPSVFLFPPKPKDTLMISRTPEVTCVVVDVSHEDPEVKFNWYVDGVEVHNAKTKPREEQYNSTYRVVSVLTVLHQDWLNGKEYKCKVSNKALPAPIEKTISKAKGQPREPQVYTLPPSRDELTKNQVSLTCLVKGFYPSDIAVEWESNGQPENNYKTTPPVLDSDGSFFLYSKLTVDKSRWQQGNVFSCSVMHEALHNHYTQKSLSLSPG

SEQ ID NO: 55 - protein, 440 aa, synthetic construct
EFGRPFVEMYSEIPEIIHMTEGRELVIPCRVTSPNITVTLKKFPLDTLIPDGKRIIWDSRKGFIISNATYKEIGLLTCEATVNGHLYKTNYLTHRQTNTIIDVQISTPSPVELCVGETLVLNCTATTPSNTRVQMTWSYPDEKNKNASVRRRIDQSNSHANIFYSVLTIDGMTNSDKGLYTCRVRSGPSFKSVNTSVHIYDCGSSGGSSGEPKSDATPTCPPCPAPELLGGPSVFLFPPKPKDTLMISRTPEVTCVVVDVSHEDPEVKFNWYVDGVEVHNAKTKPREEQYNSTYRVVSVLTVLHQDWLNGKEYKCKVSNKALPAPIEKTISKAKGQPREPQVYTLPPSRDELTKNQVSLTCLVKGFYPSDIAVEWESNGQPENNYKTTPPVLDSDGSFFLYSKLTVDKSRWQQGNVFSCSVMHEALHNHYTQKSLSLSPG

SEQ ID NO: 56 - protein, 440 aa, synthetic construct
EFGRPFVEMYSEIPEIIHMTEGRELVIPCRVTSPNITVTLKKFPLDTLIPDGKRIIWDSRKGFIISNATYKEIGLLTCEATVNGHLYKTNYLTHRQTNTIIDVQISTPSPVELCVGETLVLNCTATTPDNTRVQMTWSYPDEKNKNASVRRRIDQSNSHANIFYSVLTIDGMTNSDKGLYTCRVRSGPSFKSVNTSVHIYDCGSSGGSSGEPKSDATPTCPPCPAPELLGGPSVFLFPPKPKDTLMISRTPEVTCVVVDVSHEDPEVKFNWYVDGVEVHNAKTKPREEQYNSTYRVVSVLTVLHQDWLNGKEYKCKVSNKALPAPIEKTISKAKGQPREPQVYTLPPSRDELTKNQVSLTCLVKGFYPSDIAVEWESNGQPENNYKTTPPVLDSDGSFFLYSKLTVDKSRWQQGNVFSCSVMHEALHNHYTQKSLSLSPG

SEQ ID NO: 57 - protein, 431 aa, synthetic construct
EFGRPFVEMYSEIPEIIHMTEGRELVIPCRVTSPNITVTLKKFPLDTLIPDGKRIIWDSRKGFIISNATYKEIGLLTCEATVNGHLYKTNYLTHRQTNTIIDVQISTPSPVELCVGETLVLNCTATTPDNTRVQMTWSYPDEKNKNASVRRRIDQSNSHANIFYSVLTIDGMTNSDKGLYTCRVRSGPSFKSVNTSVHIYDCSSGDATPTSPPSPAPELLGGPSVFLFPPKPKDTLMISRTPEVTCVVVDVSHEDPEVKFNWYVDGVEVHNAKTKPREEQYNSTYRVVSVLTVLHQDWLNGKEYKCKVSNKALPAPIEKTISKAKGQPREPQVYTLPPSRDELTKNQVSLTCLVKGFYPSDIAVEWESNGQPENNYKTTPPVLDSDGSFFLYSKLTVDKSRWQQGNVFSCSVMHEALHNHYTQKSLSLSPG

SEQ ID NO: 58 - protein, 452 aa, synthetic construct
EFGRPFVEMYSEIPEIIHMTEGRELVIPCRVTSPNITVTLKKFPLDTLIPDGKRIIWDSRKGFIISNATYKEIGLLTCEATVNGHLYKTNYLTHRQTNTIIDVQISTPSPVELCVGETLVLNCTATTPDNTRVQMTWSYPDEKNKNASVRRRIDQSNSHANIFYSVLTIDGMTNSDKGLYTCRVRSGPSFKSVNTSVHIYDCSNTGSGGEEKKKEKEKEEQEERSSDTPPTCPPCPAPELLGGPSVFLFPPKPKDTLMISRTPEVTCVVVDVSHEDPEVKFNWYVDGVEVHNAKTKPREEQYNSTYRVVSVLTVLHQDWLNGKEYKCKVSNKALPAPIEKTISKAKGQPREPQVYTLPPSRDELTKNQVSLTCLVKGFYPSDIAVEWESNGQPENNYKTTPPVLDSDGSFFLYSKLTVDKSRWQQGNVFSCSVMHEALHNHYTQKSLSLSPG

SEQ ID NO: 59 - protein, 431 aa, synthetic construct
EFGRPFVEMYSEIPEIIHMTEGRELVIPCRVTSPNITVTLKKFPLDTLIPDGKRIIWDSRKGFIISNATYKEIGLLTCEATVNGHLYKTNYLTHRQTNTIIDVQISTPRPVKLLRGHTLVLNCTATTPLNTRVQMTWSYPDEKNKRASVRRRIDQSNSHANIFYSVLTIDKMQNKDKGLYTCRVRSGPSFKSVNTSVHIYDKALEDKTHTCPPCPAPELLGGPSVFLFPPKPKDTLMISRTPEVTCVVVDVSHEDPEVKFNWYVDGVEVHNAKTKPREEQYNSTYRVVSVLTVLHQDWLNGKEYKCKVSNKALPAPIEKTISKAKGQPREPQVYTLPPSRDELTKNQVSLTCLVKGFYPSDIAVEWESNGQPENNYKTTPPVLDSDGSFFLYSKLTVDKSRWQQGNVFSCSVMHEALHNHYTQKSLSLSPG

SEQ ID NO: 60 - protein, 217 aa, synthetic construct
APELLGGPSVFLFPPKPKDTLMISRTPEVTCVVVDVSHEDPEVKFNWYVDGVEVHNAKTKPREEQYNSTYRVVSVLTVLHQDWLNGKEYKCKVSNKALPAPIEKTISKAKGQPREPQVYTLPPSRDELTKNQVSLTCLVKGFYPSDIAVEWESNGQPENNYKTTPPVLDSDGSFFLYSKLTVDKSRWQQGNVFSCSVMHEALHNHYTQKSLSLSPGK

SEQ ID NO: 61 - protein, 201 aa, Homo sapiens
GRPFVEMYSEIPEIIHMTEGRELVIPCRVTSPNITVTLKKFPLDTLIPDGKRIIWDSRKGFIISNATYKEIGLLTCEATVNGHLYKTNYLTHRQTNTIIDVQISTPRPVKLLRGHTLVLNCTATTPLNTRVQMTWSYPDEKNKRASVRRRIDQSNSHANIFYSVLTIDKMQNKDKGLYTCRVRSGPSFKSVNTSVHIYDKA

SEQ ID NO: 62 - protein, 426 aa, synthetic construct
GRPFVEMYSEIPEIIHMTEGRELVIPCRVTSPNITVTLKKFPLDTLIPDGKRIIWDSRKGFIISNATYKEIGLLTCEATVNGHLYKTNYLTHRQTNTIIDVQISTPSPVTLLRGHTLVLNCTATTPLNTRVQMTWSYPDEKNKNASVRRRIDQSNSHANIFYSVLTIDKMQNKDKGLYTCRVRSGPSFKSVNTSVHIYDKDKTHTCPPCPAPELLGGPSVFLFPPKPKDTLMISRTPEVTCVVVDVSHEDPEVKFNWYVDGVEVHNAKTKPREEQYNSTYRVVSVLTVLHQDWLNGKEYKCKVSNKALPAPIEKTISKAKGQPREPQVYTLPPSREEMTKNQVSLTCLVKGFYPSDIAVEWESNGQPENNYKTTPPVLDSDGSFFLYSKLTVDKSRWQQGNVFSCSVMHEALHNHYTQKSLSLSPG

SEQ ID NO: 63 - protein, 438 aa, synthetic construct
GRPFVEMYSEIPEIIHMTEGRELVIPCRVTSPNITVTLKKFPLDTLIPDGKRIIWDSRKGFIISNATYKEIGLLTCEATVNGHLYKTNYLTHRQTNTIIDVQISTPSPVELCVGETLVLNCTATTPDNTRVQMTWSYPDEKNKNASVRRRIDQSNSHANIFYSVLTIDGMTNSDKGLYTCRVRSGPSFKSVNTSVHIYDCGSSGGSSGEPKSDATPTCPPCPAPELLGGPSVFLFPPKPKDTLMISRTPEVTCVVVDVSHEDPEVKFNWYVDGVEVHNAKTKPREEQYNSTYRVVSVLTVLHQDWLNGKEYKCKVSNKALPAPIEKTISKAKGQPREPQVYTLPPSRDELTKNQVSLTCLVKGFYPSDIAVEWESNGQPENNYKTTPPVLDSDGSFFLYSKLTVDKSRWQQGNVFSCSVMHEALHNHYTQKSLSLSPG

SEQ ID NO: 64 - protein, 438 aa, synthetic construct; identical to SEQ ID NO: 63

SEQ ID NO: 65 - protein, 450 aa, synthetic construct
GRPFVEMYSEIPEIIHMTEGRELVIPCRVTSPNITVTLKKFPLDTLIPDGKRIIWDSRKGFIISNATYKEIGLLTCEATVNGHLYKTNYLTHRQTNTIIDVQISTPSPVELCVGETLVLNCTATTPDNTRVQMTWSYPDEKNKNASVRRRIDQSNSHANIFYSVLTIDGMTNSDKGLYTCRVRSGPSFKSVNTSVHIYDCSNTGSGGEEKKKEKEKEEQEERSCDTPPTCPPCPAPELLGGPSVFLFPPKPKDTLMISRTPEVTCVVVDVSHEDPEVKFNWYVDGVEVHNAKTKPREEQYNSTYRVVSVLTVLHQDWLNGKEYKCKVSNKALPAPIEKTISKAKGQPREPQVYTLPPSRDELTKNQVSLTCLVKGFYPSDIAVEWESNGQPENNYKTTPPVLDSDGSFFLYSKLTVDKSRWQQGNVFSCSVMHEALHNHYTQKSLSLSPG

SEQ ID NO: 66 - protein, 445 aa, synthetic construct
GRPFVEMYSEIPEIIHMTEGRELVIPCRVTSPNITVTLKKFPLDTLIPDGKRIIWDSRKGFIISNATYKEIGLLTCEATVNGHLYKTNYLTHRQTNTIIDVQISTPSPVELCVGETLVLNCTATTPDNTRVQMTWSYPDEKNKNASVRRRIDQSNSHANIFYSVLTIDGMTNSDKGLYTCRVRSGPSFKSVNTSVHIYDCSGGGGSGGGGSGGGGSAESKYGPPCPPCPAPELLGGPSVFLFPPKPKDTLMISRTPEVTCVVVDVSHEDPEVKFNWYVDGVEVHNAKTKPREEQYNSTYRVVSVLTVLHQDWLNGKEYKCKVSNKALPAPIEKTISKAKGQPREPQVYTLPPSRDELTKNQVSLTCLVKGFYPSDIAVEWESNGQPENNYKTTPPVLDSDGSFFLYSKLTVDKSRWQQGNVFSCSVMHEALHNHYTQKSLSLSPG

SEQ ID NO: 67 - protein, 438 aa, synthetic construct; identical to SEQ ID NO: 63

SEQ ID NO: 68 - protein, 14 aa, synthetic construct
CSSGDATPTSPPSP

SEQ ID NO: 69 - protein, 23 aa, synthetic construct
CSKVDKKVEPKSSDTPPTCPPCP

SEQ ID NO: 70 - protein, 24 aa, synthetic construct
CSGGGGSAEPKAGDATPPTCPPCP

SEQ ID NO: 71 - protein, 30 aa, synthetic construct
CSGGGGSGGGGSGGGGSAESKYGPPCPPCP

SEQ ID NO: 72 - protein, 35 aa, synthetic construct
CSNTGSGGEEKKKEKEKEEQEERSSDTPPTCPPCP

SEQ ID NO: 73 - protein, 35 aa, synthetic construct
CSNTGSGGEEKKKEKEKEEQEERSCDTPPTCPPCP

SEQ ID NO: 74 - protein, 23 aa, synthetic construct
CGSSGGSSGEPKSDATPTCPPCP

SEQ ID NO: 75 - protein, 23 aa, synthetic construct
CSKVDKKVEPKSSDKTYTCPPCP

SEQ ID NO: 76 - protein, 33 aa, synthetic construct
NTGSGGEEKKKEKEKEEQEERSSDKTHTCPPCP

SEQ ID NO: 77 - protein, 23 aa, Homo sapiens
NTGSGGEEKKKEKEKEEQEERSS

SEQ ID NO: 78 - protein, 21 aa, synthetic construct
NTGRGGEEKKKEKEKEEQEER

SEQ ID NO: 79 - protein, 10 aa, Homo sapiens
DKTHTCPPCP